European Patent Specification EP 3 789 496 B1, published May 28, 2025. Title: A DNA-Methylation Test for Prostate Cancer. Applicant: University College Dublin, National University of Ireland, Dublin. The sequence listing filed with the application follows.

SEQUENCE LISTING (72 sequences)

SEQ ID NO: 1 - DNA, 92 bp, Homo sapiens
gctgcgcggcgactccggggactccagggcgcccctctgcggccgacgcccggggtgcagcggccgccggggctggggccggcgggagtccg

SEQ ID NO: 2 - DNA, 129 bp, Homo sapiens
agccccccggagctgcgcgcgggcttgcagcgcctcgcccgcgctgtcctcccggtgtcccgcttctccgcgccccagccgccggctgccagcttttcggggccccgagtcgcacccagcgaagagagc

SEQ ID NO: 3 - DNA, 78 bp, Homo sapiens
tttccccgacaccggctcgccgcagggagacctcaccccgagagcggaaggggtaagggcggcggggtcaaggagatc

SEQ ID NO: 4 - DNA, 77 bp, Homo sapiens
aagcgggcgtgagaccgagcgcccatgggccggtcacgccgggtgcccgctcaccccccgacgccagcaggagcgcg

SEQ ID NO: 5 - DNA, 75 bp, Homo sapiens
cggaccagggcgctccccattcccgtcgggagcccgccgattggctgggtgtgggcgcacgtgaccgacatgtgg

SEQ ID NO: 6 - DNA, 76 bp, Homo sapiens
cggaagcgctcgggcaaagactgcgaagaagaaaagacatctggcggaaacctgtgcgcctggggcggtggaactc

SEQ ID NO: 7 - DNA, 90 bp, Homo sapiens
tgggctactctggcttaacgggaccagtagcagagcgccgcccgtcctgcttgctgctgggtccggttgccgaggcggaaaagtcgcaag

SEQ ID NO: 8 - DNA, 88 bp, Homo sapiens
cctgctcctggcctctgcaggcgcctgggctgctccacctgagagctgcgcagggcggtctggcggtggctgctgcccacataatccg

SEQ ID NO: 9 - DNA, 121 bp, Homo sapiens
cgccgaggtgctgtgaccttcgtctcgccaactctctagccccagcttcatctgcaaggtgggcgggctgcttgcaaaccggtcggcgtggggtggggtcgcaccctcggctgcagcggcc

SEQ ID NO: 10 - DNA, 86 bp, Homo sapiens
gggtttcgtcgtcgttttcgttcggaggttggagtgttgttcgtcgggtcgtgcgttcgttcggtagcggcgtgtattagtattat

SEQ ID NO: 11 - DNA, 95 bp, Homo sapiens
cgctgggacgcacctgcctgttcagtcccgcaggcagaggggctgcgcctgggcctacgctcgcgatacccagaatccactcgcacctgcgaagg

SEQ ID NO: 12 - DNA, 132 bp, Homo sapiens
ctgccggaggacgcgctgctgcgagaccagccgcggcgtctttggcagtagtgggcgtgcttgcgggtccaggagggcccctctcccgcgaccgccgaccacgatgagagcgtgaagaccctctcgaaagga

SEQ ID NO: 13 - DNA, 79 bp, Homo sapiens
cggtcctggctcaaactctcgtcacctgatcctcggcgaaagctcctatcgcgacactttgaccgtagccgttcccgcc

SEQ ID NO: 14 - DNA, 135 bp, Homo sapiens
acgtgtggcctgtcacaccgtcggctgtattggatcaggattatttcttatgaaggtctgctttgccagtacgcagcaggtcccagtctctacgccgtcccgaacacctcgtagaaatacggggcatgcacaacg

SEQ ID NO: 15 - DNA, 101 bp, Homo sapiens
cggattccgttcatgcctctcggagctacagggcttggtgcggagacgcagggcgggcgcgctgggctctgggtgtccgcaacccaaagtgcagctggtgt

SEQ ID NO: 16 - DNA, 100 bp, Homo sapiens
cgggtcgcctccacctcccgcagccgccgcgccccggctcgccgcgctcccgccggcaccatggaggaattcctgggacaaccgcctgcagccggcgact

SEQ ID NO: 17 - DNA, 98 bp, Homo sapiens
ggtggaggcagccagggcttacctgtacactgacttgagaccagttgaataaaagtgcacaccttaaaaatgaggccaagtgtgactttgtggtgtgg

SEQ ID NO: 18 - DNA, 1335 bp, Homo sapiens
agccccaagcttaccacctgcacccggagagctgtgtcaccatgtgggtcccggttgtcttcctcaccctgtccgtgacgtggattggtgctgcacccctcatcctgtctcggattgtgggaggctgggagtgcgagaagcattcccaaccctggcaggtgcttgtggcctctcgtggcagggcagtctgcggcggtgttctggtgcacccccagtgggtcctcacagctgcccactgcatcaggaagccaggtgatgactccagccacgacctcatgctgctccgcctgtcagagcctgccgagctcacggatgctgtgaaggtcatggacctgcccacccaggagccagcactggggaccacctgctacgcctcaggctggggcagcattgaaccagaggagttcttgaccccaaagaaacttcagtgtgtggacctccatgttatttccaatgacgtgtgtgcgcaagttcaccctcagaaggtgaccaagttcatgctgtgtgctggacgctggacagggggcaaaagcacctgctcgggtgattctgggggcccacttgtctgtaatggtgtgcttcaaggtatcacgtcatggggcagtgaaccatgtgccctgcccgaaaggccttccctgtacaccaaggtggtgcattaccggaagtggatcaaggacaccatcgtggccaacccctgagcacccctatcaaccccctattgtagtaaacttggaaccttggaaatgaccaggccaagactcaagcctccccagttctactgacctttgtccttaggtgtgaggtccagggttgctaggaaaagaaatcagcagacacaggtgtagaccagagtgtttcttaaatggtgtaattttgtcctctctgtgtcctggggaatactggccatgcctggagacatatcactcaatttctctgaggacacagataggatggggtgtctgtgttatttgtggggtacagagatgaaagaggggtgggatccacactgagagagtggagagtgacatgtgctggacactgtccatgaagcactgagcagaagctggaggcacaacgcaccagacactcacagcaaggatggagctgaaaacataacccactctgtcctggaggcactgggaagcctagagaaggctgtgagccaaggagggagggtcttcctttggcatgggatggggatgaagtaaggagagggactggaccccctggaagctgattcactatggggggaggtgtattgaagtcctccagacaaccctcagatttgatgatttcctagtagaactcacagaaataaagagctgttatactgtg

SEQ ID NO: 19 - DNA, 648 bp, Artificial Sequence
  Synthetic Block Sequence
aaaggtggaggtagttagggtttatttgtatattgatttgagattagttgaataaaagtgtatattttaaaaatgaggttaagtgtgattttgtggtgtggaaagttgcgcggcgatttcggggattttagggcgtttttttgcggtcgacgttcggggtgtagcggtcgtcggggttggggtcggcgggagttcgaaaagtttttcggagttgcgcgcgggtttgtagcgtttcgttcgcgttgttttttcggtgtttcgttttttcgcgttttagtcgtcggttgttagtttttcggggtttcgagtcgtatttagcgaagagagcaaattttttcgatatcggttcgtcgtagggagattttatttcgagagcggaaggggtaagggcggcggggttaaggagatcaaaaagcgggcgtgagatcgagcgtttatgggtcggttacgtcgggtgttcgtttatttttcgacgttagtaggagcgcgaaattatatgtcggttacgtgcgtttatatttagttaatcggcgggttttcgacgggaatggggagcgttttggttcaaacggaagcgttcgggtaaagattgcgaagaagaaaagatatttggcggaaatttgtgcgtttggggcggtggaattcaaa

SEQ ID NO: 20 - DNA, 885 bp, Artificial Sequence
  Synthetic Block Sequence
aaaggtggaggtagttagggtttatttgtatattgatttgagattagttgaataaaagtgtatattttaaaaatgaggttaagtgtgattttgtggtgtggaaatgggttattttggtttaacgggattagtagtagagcgtcgttcgttttgtttgttgttgggttcggttgtcgaggcggaaaagtcgtaagaaatttgtttttggtttttgtaggcgtttgggttgttttatttgagagttgcgtagggcggtttggcggtggttgttgtttatataattcgaaacgtcgaggtgttgtgattttcgtttcgttaattttttagttttagttttatttgtaaggtgggcgggttgtttgtaaatcggtcggcgtggggtggggtcgtattttcggttgtagcggttaaagggtttcgtcgtcgttttcgttcggaggttggagtgttgttcgtcgggtcgtgcgttcgttcggtagcggcgtgtattagtattataaacgttgggacgtatttgtttgtttagtttcgtaggtagaggggttgcgtttgggtttacgttcgcgatatttagaatttattcgtatttgcgaaggcgaaaatacgtttttgtcggtcgtttagttttttgtaggtgtaagggcggatgttttagcgattacgggagtcgggttggggaggttggtggggggcggggggagttttaaatttaggttcgtttagttataggcgtttaggtttagtcggaaattgtcggaggacgcgttgttgcgagattagtcgcggcgtttttggtagtagtgggcgtgtttgcgggtttaggagggtttttttttcgcgatcgtcgattacgatgagagcgtgaagattttttcgaaaggaaaa

SEQ ID NO: 21 - DNA, 643 bp, Artificial Sequence
  Synthetic Block Sequence
aaagggcggttttggtttaaattttcgttatttgattttcggcgaaagtttttatcgcgatattttgatcgtagtcgttttcgttaaaaaaggtggaggtagttagggtttatttgtatattgatttgagattagttgaataaaagtgtatattttaaaaatgaggttaagtgtgattttgtggtgtggaaattcggtttattacggcggttatttttcgggtagtgacgacgatcgagacggtgagggcggttatcgttggggagggaggttcgggtttaggtttggaagtaaaacgtgtggtttgttatatcgtcggttgtattggattaggattattttttatgaaggtttgttttgttagtacgtagtaggttttagtttttacgtcgtttcgaatatttcgtagaaatacggggtatgtataacgaaacggatttcgtttatgtttttcggagttatagggtttggtgcggagacgtagggcgggcgcgttgggttttgggtgttcgtaatttaaagtgtagttggtgtaaacgggtcgtttttatttttcgtagtcgtcgcgtttcggttcgtcgcgttttcgtcggtattatggaggaatttttgggataatcgtttgtagtcggcgattgggaaa

SEQ ID NO: 22 - DNA, 27 bp, Artificial Sequence
  Primer ACTB
ggtggaggtagttagggtttatttgta

SEQ ID NO: 23 - DNA, 30 bp, Artificial Sequence
  Primer ACTB
ccacaccacaaaatcacacttaacctcatt

SEQ ID NO: 24 - DNA, 17 bp, Artificial Sequence
  Primer GSTP1
gttgcgtggcgatttcg

SEQ ID NO: 25 - DNA, 16 bp, Artificial Sequence
  Primer GSTP1
cgaactcccgccgacc

SEQ ID NO: 26 - DNA, 19 bp, Artificial Sequence
  Primer SFRP2
agtttttcggagttgcgcg

SEQ ID NO: 27 - DNA, 24 bp, Artificial Sequence
  Primer SFRP2
gctctcttcgctaaatacgactcg

SEQ ID NO: 28 - DNA, 22 bp, Artificial Sequence
  Primer IGFBP3
ttttttcgatatcggttcgtcg

SEQ ID NO: 29 - DNA, 19 bp, Artificial Sequence
  Primer IGFBP3
gatctccttaaccccgccg

SEQ ID NO: 30 - DNA, 17 bp, Artificial Sequence
  Primer IGFBP7
aagcgggcgtgagatcg

SEQ ID NO: 31 - DNA, 19 bp, Artificial Sequence
  Primer IGFBP7
cgcgctcctactaacgtcg

SEQ ID NO: 32 - DNA, 27 bp, Artificial Sequence
  Primer APC
ttatatgtccgttacgtgcgtttatat

SEQ ID NO: 33 - DNA, 19 bp, Artificial Sequence
  Primer APC
gaaccaaaacgctccccat

SEQ ID NO: 34 - DNA, 19 bp, Artificial Sequence
  Primer PTGS2
cggaagcgttcgggtaaag

SEQ ID NO: 35 - DNA, 20 bp, Artificial Sequence
  Primer PTGS2
gaattccaccgccccaaacg

SEQ ID NO: 36 - DNA, 22 bp, Artificial Sequence
  Primer LXN
tgggttattttggtttaacggg

SEQ ID NO: 37 - DNA, 20 bp, Artificial Sequence
  Primer LXN
cttacgacttttccgcctcg

SEQ ID NO: 38 - DNA, 23 bp, Artificial Sequence
  Primer MAGPIE-1
tttgtttttggtttttgtaggcg

SEQ ID NO: 39 - DNA, 25 bp, Artificial Sequence
  Primer MAGPIE-1
cgaattatataaacaacaaccaccg

SEQ ID NO: 40 - DNA, 20 bp, Artificial Sequence
  Primer DNAH10
cgtcgaggtgttgtgatttt

SEQ ID NO: 41 - DNA, 22 bp, Artificial Sequence
  Primer DNAH10
aaccgctacaaccgaaaatacg

SEQ ID NO: 42 - DNA, 17 bp, Artificial Sequence
  Primer ZMIZ1
gggtttcgtcgtcgttt

SEQ ID NO: 43 - DNA, 22 bp, Artificial Sequence
  Primer ZMIZ1
ataatactaatacacgccgcta

SEQ ID NO: 44 - DNA, 21 bp, Artificial Sequence
  Primer CENPV
cgttgggacgtatttgtttgt

SEQ ID NO: 45 - DNA, 20 bp, Artificial Sequence
  Primer CENPV
cgccttcgcaaatacgaata

SEQ ID NO: 46 - DNA, 17 bp, Artificial Sequence
  Primer OR2L13
ttgtcggaggacgcgtt

SEQ ID NO: 47 - DNA, 23 bp, Artificial Sequence
  Primer OR2L13
tcctttcgaaaaaatcttcacgc

SEQ ID NO: 48 - DNA, 24 bp, Artificial Sequence
  Primer MTMR8
cgggtttttattttcgttttttcg

SEQ ID NO: 49 - DNA, 24 bp, Artificial Sequence
  Primer MTMR8
aaaataacgtagtcgttttcgatc

SEQ ID NO: 50 - DNA, 21 bp, Artificial Sequence
  Primer F3
tgtggtttgttatatcgtcgg

SEQ ID NO: 51 - DNA, 23 bp, Artificial Sequence
  Primer F3
aatacaacgttatacataccccg

SEQ ID NO: 52 - DNA, 23 bp, Artificial Sequence
  Primer CDH8
cggatttcgtttatgtttttcgg

SEQ ID NO: 53 - DNA, 24 bp, Artificial Sequence
  Primer CDH8
acaccaactacactttaaattacg

SEQ ID NO: 54 - DNA, 23 bp, Artificial Sequence
  Primer GALNTL6
cgggtcgtttttatttttcgtag

SEQ ID NO: 55 - DNA, 18 bp, Artificial Sequence
  Primer GALNTL6
aatcgccgactacaaacg

SEQ ID NO: 56 - DNA, 21 bp, Artificial Sequence
  Probe ACTB
cacttttattcaactaatctc

SEQ ID NO: 57 - DNA, 15 bp, Artificial Sequence
  Probe GSTP1
cgacgaccgctacac

SEQ ID NO: 58 - DNA, 17 bp, Artificial Sequence
  Probe SFRP2
tgtagcgtttcgttcgc

SEQ ID NO: 59 - DNA, 21 bp, Artificial Sequence
  Probe IFGBP3
agattttatttcgagagcgga

SEQ ID NO: 60 - DNA, 19 bp, Artificial Sequence
  Probe IGFBP7
ttatgggtcggttacgtcg

SEQ ID NO: 61 - DNA, 22 bp, Artificial Sequence
  Probe APC
cccgtcgaaaacccgccgatta

SEQ ID NO: 62 - DNA, 29 bp, Artificial Sequence
  Probe PTGS2
tttccgccaaatatcttttcttcttcgca

SEQ ID NO: 63 - DNA, 27 bp, Artificial Sequence
  Probe LXN
cgtcgttcgttttgtttgttgttgggt

SEQ ID NO: 64 - DNA, 22 bp, Artificial Sequence
  Probe MAGPIE-1
tttgagagttgcgtagggcggt

SEQ ID NO: 65 - DNA, 25 bp, Artificial Sequence
  Probe DNAH10
cgggttgtttgtaaatcggtcggcg

SEQ ID NO: 66 - DNA, 24 bp, Artificial Sequence
  Probe ZMIZ1
ttcggaggttggagtgttgttcgt

SEQ ID NO: 67 - DNA, 24 bp, Artificial Sequence
  Probe CENPV
ttgcgtttgggtttacgttcgcga

SEQ ID NO: 68 - DNA, 25 bp, Artificial Sequence
  Probe OR2L13
tgcgagattagtcgcggcgtttttg

SEQ ID NO: 69 - DNA, 27 bp, Artificial Sequence
  Probe MTMR8
tgattttcggcgaaagtttttatcgcg

SEQ ID NO: 70 - DNA, 31 bp, Artificial Sequence
  Probe F3
cgtagtaggttttagtttttacgtcgtttcg

SEQ ID NO: 71 - DNA, 17 bp, Artificial Sequence
  Probe CDH8
cgtagggcgggcgcgtt

SEQ ID NO: 72 - DNA, 19 bp, Artificial Sequence
  Probe GALNTL6
cgcgtttcggttcgtcgcg